European Patent Application EP 4 800 034 A1, published September 2, 2026. Title: 225Ac-labeled anti-CDH3 antibody. Applicant: 株式会社ペルセウスプロテオミクス. Application JP, filed October 25, 2024. The sequence listing filed with the application follows.

SEQUENCE LISTING (10 sequences)

SEQ ID NO: 1 - protein, 449 aa, synthetic construct
  source 1..449: note = heavy chain of FF-21101
EVKLEESGPELVKPGDSVKMSCKASGYTFTDYYIDWVKQSHGKSLEWIGYIYPNNGGTNYNQKFKGKATLTVDKSSSTAYMELHSLTSEDSAVYYCARSGGAPHFDYWGQGTTLTVSSASTKGPSVFPLAPSSKSTSGGTAALGCLVKDYFPEPVTVSWNSGALTSGVHTFPAVLQSSGLYSLSSVVTVPSSSLGTQTYICNVNHKPSNTKVDKKVEPPKSCDKTHTCPPCPAPELLGGPSVFLFPPKPKDTLMISRTPEVTCVVVDVSHEDPEVKFNWYVDGVEVHNAKTKPREEQYNSTYRVVSVLTVLHQDWLNGKEYKCKVSNKALPAPIEKTISKAKGQPREPQVYTLPPSRDELTKNQVSLTCLVKGFYPSDIAVEWESNGQPENNYKTTPPVLDSDGSFFLYSKLTVDKSRWQQGNVFSCSVMHEALHNHYTQKSLSLSPGK

SEQ ID NO: 2 - protein, 218 aa, synthetic construct
  source 1..218: note = light chain of FF-21101
DIVLTQSPASLTVSLGQRATISCRASISVSTSSYSFMHWFQQKPGQPPKLLIRYASYLESGVPARFSGSGSGTDFTLNIHPVEEEDAATYYCQHSREFPRTFGGGTKLEIKRTVAAPSVFIFPPSDEQLKSGTASVVCLLNNFYPREAKVQWKVDNALQSGNSQESVTEQDSKDSTYSLSSTLTLSKADYEKHKVYACEVTHQGLSSPVTKSFNRGEC

SEQ ID NO: 3 - protein, 5 aa, synthetic construct
  source 1..5: note = heavy chain CDR1
DYYID

SEQ ID NO: 4 - protein, 17 aa, synthetic construct
  source 1..17: note = heavy chain CDR2
YIYPNNGGTNYNQKFKG

SEQ ID NO: 5 - protein, 9 aa, synthetic construct
  source 1..9: note = heavy chain CDR3
SGGAPHFDY

SEQ ID NO: 6 - protein, 15 aa, synthetic construct
  source 1..15: note = light chain CDR1
RASISVSTSSYSFMH

SEQ ID NO: 7 - protein, 7 aa, synthetic construct
  source 1..7: note = light chain CDR2
YASYLES

SEQ ID NO: 8 - protein, 9 aa, synthetic construct
  source 1..9: note = light chain CDR3
QHSREFPRT

SEQ ID NO: 9 - protein, 118 aa, synthetic construct
  source 1..118: note = heavy chain variable region
EVKLEESGPELVKPGDSVKMSCKASGYTFTDYYIDWVKQSHGKSLEWIGYIYPNNGGTNYNQKFKGKATLTVDKSSSTAYMELHSLTSEDSAVYYCARSGGAPHFDYWGQGTTLTVSS

SEQ ID NO: 10 - protein, 111 aa, synthetic construct
  source 1..111: note = light chain variable region
DIVLTQSPASLTVSLGQRATISCRASISVSTSSYSFMHWFQQKPGQPPKLLIRYASYLESGVPARFSGSGSGTDFTLNIHPVEEEDAATYYCQHSREFPRTFGGGTKLEIK